European Patent Application EP 4 382 127 A2, published June 12, 2024. Title: GLYPICAN 2 AS A CANCER MARKER AND THERAPEUTIC TARGET. Applicant: The Children's Hospital of Philadelphia The Government of the United States of America as represented by the Secretary of the Department of Health and Human Services. Application EP. The sequence listing filed with the application follows.

SEQUENCE LISTING (30 sequences)

SEQ ID NO: 1 - DNA, 357 bp, synthetic construct
  misc_feature 1..357: note = Synthetic oligonucleotide
  source 1..357: mol_type = other DNA
gaggtgcagctggtggagactgggggaggcgtggtcaagcctggagggtccctgagactctcctgtgcagcctctggattcaccttcagtgactactacatgagctggatccgccaggctccagggaaggggctggagtgggtttcatacattagtagtagtggtagtaccatatactacgcagactccgtgaagggccgattcaccatctccagagacaattccaagaacacgctgtatctgcaaatgaacagcctgagagctgaggacacggctgtgtattactgtgcgagagagagtggctacgattacgtgtttgactactggggccagggaaccctggtcgccgtctcctca

SEQ ID NO: 2 - protein, 119 aa, synthetic construct
  REGION 1..119: note = Synthetic amino acid
EVQLVETGGGVVKPGGSLRLSCAASGFTFSDYYMSWIRQAPGKGLEWVSYISSSGSTIYYADSVKGRFTISRDNSKNTLYLQMNSLRAEDTAVYYCARESGYDYVFDYWGQGTLVAVSS

SEQ ID NO: 3 - DNA, 324 bp, synthetic construct
  misc_feature 1..324: note = Synthetic oligonucleotide
  source 1..324: mol_type = other DNA
gacatccagatgacccagtctccttccaccctgtctgcatttgtaggagacagagtcaccatcacttgccgggccagtcagagtattagtagctggttggcctggtatcagcaaaaaccagggaaagcccctaagctcctgatctatgctgcatccactttgcaaagtggggtcccatcaaggttcagcggcagtggatctgggacagaattcactctcacaatcagcagcctgcagcctgaagattttgcaacttattactgtcaacagcttaatagttaccctatcaccttcggccaagggacacgactggagattaaacga

SEQ ID NO: 4 - protein, 108 aa, synthetic construct
  REGION 1..108: note = Synthetic amino acid
DIQMTQSPSTLSAFVGDRVTITCRASQSISSWLAWYQQKPGKAPKLLIYAASTLQSGVPSRFSGSGSGTEFTLTISSLQPEDFATYYCQQLNSYPITFGQGTRLEIKR

SEQ ID NO: 5 - protein, 8 aa, synthetic construct
  REGION 1..8: note = Synthetic amino acid
GFTFSDYY

SEQ ID NO: 6 - protein, 8 aa, synthetic construct
  REGION 1..8: note = Synthetic amino acid
ISSSGSTI

SEQ ID NO: 7 - protein, 12 aa, synthetic construct
  REGION 1..12: note = Synthetic amino acid
ARESGYDYVFDY

SEQ ID NO: 8 - protein, 6 aa, synthetic construct
  REGION 1..6: note = Synthetic amino acid
QSISSW

SEQ ID NO: 9 - skipped

SEQ ID NO: 10 - protein, 9 aa, synthetic construct
  REGION 1..9: note = Synthetic amino acid
QQLNSYPIT

SEQ ID NO: 11 - DNA, 345 bp, synthetic construct
  misc_feature 1..345: note = Synthetic oligonucleotide
  source 1..345: mol_type = other DNA
caggtgcagctggtgcagtctggaggaggcttgatccagcctggggggtccctgagactctcctgtgcagcctctgggttcaccgtcagtagcaactacatgagctgggtccgccaggctccagggaaggggctggagtgggtctcagttatttatagcggtggtagcacatactacgcagactccgtgaagggccgattcaccatctccagagacaattccaagaacacgctgtatcttcaaatgaacagcctgagagccgaggacacggccgtgtattactgtgcgagagattcgaatgcttttgatatctggggccaagggacaatggtcaccgtctcttca

SEQ ID NO: 12 - protein, 115 aa, synthetic construct
  REGION 1..115: note = Synthetic amino acid
QVQLVQSGGGLIQPGGSLRLSCAASGFTVSSNYMSWVRQAPGKGLEWVSVIYSGGSTYYADSVKGRFTISRDNSKNTLYLQMNSLRAEDTAVYYCARDSNAFDIWGQGTMVTVSS

SEQ ID NO: 13 - DNA, 339 bp, synthetic construct
  misc_feature 1..339: note = Synthetic oligonucleotide
  source 1..339: mol_type = other DNA
gaaattgtgctgactcagtctccactctccctgcccgtcacccctggagagccggcctccatctcctgcaggtctagtcagagcctcctgtatagtaatggatacaactatttggattggtacctgcagaagccagggaagtctccacaggtcctgatctatttgggttctaatcgggcctccggggtccccgacaggttcagtggcagtggatcaggcacagatttcacactgaaaatcagcagagtggaggctgaggatgttggggtttattactgcatgcaagctctacaaactccgatcaccttcggccaagggacacgactggagattaaacga

SEQ ID NO: 14 - protein, 113 aa, synthetic construct
  REGION 1..113: note = Synthetic amino acid
EIVLTQSPLSLPVTPGEPASISCRSSQSLLYSNGYNYLDWYLQKPGKSPQVLIYLGSNRASGVPDRFSGSGSGTDFTLKISRVEAEDVGVYYCMQALQTPITFGQGTRLEIKR

SEQ ID NO: 15 - protein, 8 aa, synthetic construct
  REGION 1..8: note = Synthetic amino acid
GFTVSSNY

SEQ ID NO: 16 - protein, 8 aa, synthetic construct
  REGION 1..8: note = Synthetic amino acid
VIYSGGST

SEQ ID NO: 17 - protein, 9 aa, synthetic construct
  REGION 1..9: note = Synthetic amino acid
ARDSNAFDI

SEQ ID NO: 18 - protein, 11 aa, synthetic construct
  REGION 1..11: note = Synthetic amino acid
QSLLYSNGYNY

SEQ ID NO: 19 - skipped

SEQ ID NO: 20 - protein, 9 aa, synthetic construct
  REGION 1..9: note = Synthetic amino acid
MQALQTPIT

SEQ ID NO: 21 - DNA, 366 bp, synthetic construct
  misc_feature 1..366: note = Synthetic oligonucleotide
  source 1..366: mol_type = other DNA
gaggtgcagctggtgcagtctgggggaggcttggtacagcctggggggtccctgagactctcctgtgcagcctctggattcacctttagcagctatgccatgagctgggtccgccaggctccagggaaggggctggagtgggtctcagctattagtggtagtggtggtagcacatactacgcagactccgtgaagggccgcttcaccatctccagagacaattccaagaacacgctgtctctgcaaatggacagcctgagacccgaggacacggccgtatattactgtgcgaaaagtcgagatagtgggaactaccttgatgcttttgatttctggggccaagggacaatggtcaccgtctcttca

SEQ ID NO: 22 - protein, 122 aa, synthetic construct
  REGION 1..122: note = Synthetic amino acid
EVQLVQSGGGLVQPGGSLRLSCAASGFTFSSYAMSWVRQAPGKGLEWVSAISGSGGSTYYADSVKGRFTISRDNSKNTLSLQMDSLRPEDTAVYYCAKSRDSGNYLDAFDFWGQGTMVTVSS

SEQ ID NO: 23 - DNA, 324 bp, synthetic construct
  misc_feature 1..324: note = Synthetic oligonucleotide
  source 1..324: mol_type = other DNA
gacatccagttgacccagtctccttccaccctgtctgcatctgtaggagacagagtcaccatcacttgccgggccagtcagagtattagtagctggttggcctggtatcagcagaaagcagggaaagctcctaggctcctgatctatgatgcctccactttggaaagtggagtcccatcaaggttcagcggcactggatctgggacatatttcactctcaccatcagcagcctgcagcctgaagattttgcaacttattactgtcaacagtttaatagtttcccgctcactttcggcggagggaccaaggtggagatcaaacga

SEQ ID NO: 24 - protein, 108 aa, synthetic construct
  REGION 1..108: note = Synthetic amino acid
DIQLTQSPSTLSASVGDRVTITCRASQSISSWLAWYQQKAGKAPRLLIYDASTLESGVPSRFSGTGSGTYFTLTISSLQPEDFATYYCQQFNSFPLTFGGGTKVEIKR

SEQ ID NO: 25 - protein, 8 aa, synthetic construct
  REGION 1..8: note = Synthetic amino acid
GFTFSSYA

SEQ ID NO: 26 - protein, 8 aa, synthetic construct
  REGION 1..8: note = Synthetic amino acid
ISGSGGST

SEQ ID NO: 27 - protein, 15 aa, synthetic construct
  REGION 1..15: note = Synthetic amino acid
AKSRDSGNYLDAFDF

SEQ ID NO: 28 - protein, 6 aa, synthetic construct
  REGION 1..6: note = Synthetic amino acid
QSISSW

SEQ ID NO: 29 - skipped

SEQ ID NO: 30 - protein, 9 aa, synthetic construct
  REGION 1..9: note = Synthetic amino acid
QQFNSFPLT